European Patent Specification EP 3 546 580 B1, published September 3, 2025. Title: VECTORS FOR TRANSFORMING MYCOPLASMA HYOPNEUMONIAE, TRANSFORMED M.HYOPNEUMONIAE STRAINS, AND USE THEREOF. Applicant: Laboratorios Hipra, S.L.U. Application not yet assigned. The sequence listing filed with the application follows.

SEQUENCE LISTING (45 sequences)

SEQ ID NO: 1 - DNA, 265 bp, Mycoplasma hyopneumoniae
gaagactgattagaaatttagaactattcaaatctttcaaaaaagtggcctaaaaacaatgataaaaaaatttccaaacttttttgttgcaaaaaaaaaaaaaaaaagtataattttaattgtacaagttaaataaatttttcacttatctttttttattttgcaaaacttttaaaaaaattagatatctaaattatattatatgattgagaaaatgaaaaatttatttcctagaaccaagataattgaggtttaaaatatgagt

SEQ ID NO: 2 - DNA, 263 bp, Mycoplasma hyopneumoniae
ttgaatttgtattttccataatctaaaattttacatttttttataacaatttttaaaaattaccctttaatttatagtatttttttattttttagtctaaattataaaattatcttgaattttatttgaatttttataatttagtactaaaaaatacaaatattttttcctattctaagaaaaattcattttttaaaaaaaattgatttttatagtataatttatttgtataattgaattaacttgatttgaaagggaacaaa

SEQ ID NO: 3 - DNA, 699 bp, Artificial Sequence
  synthetic gene
atgacatatccaagaagaagatatagaagaagaagacatagaccaagatcacatttaggacaaattttaagaagaagaccatgattagttcatccaagacatagatatagatgaagaagaaaaaatggaatttttaatacaagattatcaagaacatttggatatacagttaaaagaacaacagttacaacaccatcatgagcagttgatatgatgagatttaaaattgatgattttgttccaccaggaggaggaacaaataaaatttcaattccatttgaatattatagaattagaaaagttaaagttgaattttgaccatgttcaccaattacacaaggagatagaggagttggatcaacagcagttattttagatgataattttgttacaaaagcaacagcattaacatatgatccatatgttaattattcatcaagacatacaattccacaaccattttcatatcattcaagatattttacaccaaaaccagttttagattcaacaattgattattttcaaccaaataataaaagaaatcaattatgattaagattacaaacatcaggaaatgttgatcatgttggattaggaacagcatttgaaaattcaaaatatgatcaagattataatattagagttacaatgtatgttcaatttagagaatttaatttaaaagatccaccattagaacca

SEQ ID NO: 4 - DNA, 702 bp, Artificial Sequence
  synthetic gene
atgacatatccaagaagaagatatagaagaagaagacatagaccaagatcacatttaggacaaattttaagaagaagaccatgattagttcatccaagacatagatatagatgaagaagaaaaaatggaatttttaatacaagattatcaagaacatttggatatacagttaaaagaacaacagttacaacaccatcatgagcagttgatatgatgagatttaaaattgatgattttgttccaccaggaggaggaacaaataaaatttcaattccatttgaatattatagaattagaaaagttaaagttgaattttgaccatgttcaccaattacacaaggagatagaggagttggatcaacagcagttattttagatgataattttgttacaaaagcaacagcattaacatatgatccatatgttaattattcatcaagacatacaattccacaaccattttcatatcattcaagatattttacaccaaaaccagttttagattcaacaattgattattttcaaccaaataataaaagaaatcaattatgattaagattacaaacatcaggaaatgttgatcatgttggattaggaacagcatttgaaaattcaaaatatgatcaagattataatattagagttacaatgtatgttcaatttagagaatttaatttaaaagatccaccattagaaccataa

SEQ ID NO: 5 - DNA, 992 bp, Artificial Sequence
  synthetic gene
actagtactagagaagactgattagaaatttagaactattcaaatctttcaaaaaagtggcctaaaaacaatgataaaaaaatttccaaacttttttgttgcaaaaaaaaaaaaaaaagtataattttaattgtacaagttaaataaatttttcacttatctttttttattttgcaaaacttttaaaaaaattagatatctaaattatattatatgattgagaaaatgaaaaatttatttcctagaaccaagataattgaggtttaaaatatgagtggatccatgacatatccaagaagaagatatagaagaagaagacatagaccaagatcacatttaggacaaattttaagaagaagaccatgattagttcatccaagacatagatatagatgaagaagaaaaaatggaatttttaatacaagattatcaagaacatttggatatacagttaaaagaacaacagttacaacaccatcatgagcagttgatatgatgagatttaaaattgatgattttgttccaccaggaggaggaacaaataaaatttcaattccatttgaatattatagaattagaaaagttaaagttgaattttgaccatgttcaccaattacacaaggagatagaggagttggatcaacagcagttattttagatgataattttgttacaaaagcaacagcattaacatatgatccatatgttaattattcatcaagacatacaattccacaaccattttcatatcattcaagatattttacaccaaaaccagttttagattcaacaattgattattttcaaccaaataataaaagaaatcaattatgattaagattacaaacatcaggaaatgttgatcatgttggattaggaacagcatttgaaaattcaaaatatgatcaagattataatattagagttacaatgtatgttcaatttagagaatttaatttaaaagatccaccattagaaccataagcggccgc

SEQ ID NO: 6 - protein, 233 aa, Porcine circovirus type 2 (PCV2)
MTYPRRRYRRRRHRPRSHLGQILRRRPWLVHPRHRYRWRRKNGIFNTRLSRTFGYTVKRTTVTTPSWAVDMMRFKIDDFVPPGGGTNKISIPFEYYRIRKVKVEFWPCSPITQGDRGVGSTAVILDDNFVTKATALTYDPYVNYSSRHTIPQPFSYHSRYFTPKPVLDSTIDYFQPNNKRNQLWLRLQTSGNVDHVGLGTAFENSKYDQDYNIRVTMYVQFREFNLKDPPLEP

SEQ ID NO: 7 - DNA, 26 bp, Staphylococcus aureus
gataaagtccgtataattgtgtaaaa

SEQ ID NO: 8 - DNA, 26 bp, Staphylococcus aureus
ttttacacaattatacggactttatc

SEQ ID NO: 9 - DNA, 33 bp, Artificial Sequence
  primer
atgcgcggccgcttatttatcagaaacagttag

SEQ ID NO: 10 - DNA, 38 bp, Artificial Sequence
  primer
agtcgggcccagcttgcgcatcattggatgatggattc

SEQ ID NO: 11 - DNA, 29 bp, Artificial Sequence
  primer
actgggatccatgaatatagttgaaaatg

SEQ ID NO: 12 - DNA, 27 bp, Artificial Sequence
  primer
ggatgggcccagcttgcgcatcattgg

SEQ ID NO: 13 - DNA, 40 bp, Artificial Sequence
  primer
gatctctagatcgaggaagactgattagaaatttagaact

SEQ ID NO: 14 - DNA, 34 bp, Artificial Sequence
  primer
gatcggatccactcatattttaaacctcaattat

SEQ ID NO: 15 - DNA, 27 bp, Artificial Sequence
  primer
actgactagtagcttgcgcatcattgg

SEQ ID NO: 16 - DNA, 43 bp, Artificial Sequence
  primer
atgcagatctatgtccaatttactgaccgtacaccaaaatttg

SEQ ID NO: 17 - DNA, 37 bp, Artificial Sequence
  primer
atgcgggcccttaatcgccatcttccagcaggcgcac

SEQ ID NO: 18 - DNA, 45 bp, Artificial Sequence
  primer
tgttatcgataccgtcgatgcacctcgagctaagttattttattg

SEQ ID NO: 19 - DNA, 44 bp, Artificial Sequence
  primer
agacatcgaaagcttgattatgctgattgcattctttcaatttg

SEQ ID NO: 20 - DNA, 42 bp, Artificial Sequence
  primer
agaggaatccgatttatttatcagaaacagttagtcttttcc

SEQ ID NO: 21 - DNA, 58 bp, Artificial Sequence
  primer
agactctagaactagtggatcccccgggcccctcgaggaagactgattagaaatttag

SEQ ID NO: 22 - DNA, 46 bp, Artificial Sequence
  primer
agacgaattcgaattcctgcagggatccactcatattttaaacctc

SEQ ID NO: 23 - DNA, 34 bp, Artificial Sequence
  primer
catcgaattcacgaattagtgattctgccttttc

SEQ ID NO: 24 - DNA, 35 bp, Artificial Sequence
  primer
catcgaattcattaaagttgattcggtgtttaatc

SEQ ID NO: 25 - DNA, 35 bp, Artificial Sequence
  primer
catgctgcagcccgggggatccactagttctagag

SEQ ID NO: 26 - DNA, 27 bp, Artificial Sequence
  primer
gtacccaattcgccctatagtgagtcg

SEQ ID NO: 27 - DNA, 30 bp, Artificial Sequence
  primer
tcgaggaagactgattagaaatttagaact

SEQ ID NO: 28 - DNA, 40 bp, Artificial Sequence
  primer
gatcgggccctcgaggaagactgattagaaatttagaact

SEQ ID NO: 29 - DNA, 39 bp, Artificial Sequence
  primer
gatcggatccatgacccaagtacattttacactgaaaag

SEQ ID NO: 30 - DNA, 39 bp, Artificial Sequence
  primer
gatcctcgagggggggcccttttacacaattatacggac

SEQ ID NO: 31 - DNA, 34 bp, Artificial Sequence
  primer
gatcggatccatgaaaattattaatattggagtt

SEQ ID NO: 32 - DNA, 50 bp, Artificial Sequence
  primer
gatcgctgcaggaattcgatatcaagcttatcgataccgtcgatgcacct

SEQ ID NO: 33 - DNA, 34 bp, Artificial Sequence
  primer
ataacttcgtatagcatacattatacgaacggta

SEQ ID NO: 34 - DNA, 69 bp, Artificial Sequence
  primer
gattaagggcccataacttcgtataggatactttatacgaagttatgtcgaccccctcgaggaagactg

SEQ ID NO: 35 - DNA, 74 bp, Artificial Sequence
  primer
gggactagttacggttcgtataatgtatgctatacgaagttatctgcaggatatcaagcttatcgataccgtcg

SEQ ID NO: 36 - DNA, 34 bp, Artificial Sequence
  primer
gtgtaagcttaaaaaccaggatgcacaaaataac

SEQ ID NO: 37 - DNA, 34 bp, Artificial Sequence
  primer
tgttgcggccgctttaggcatcaggattatcaac

SEQ ID NO: 38 - DNA, 33 bp, Artificial Sequence
  primer
agacactagtttgaatttgtattttccataatc

SEQ ID NO: 39 - DNA, 33 bp, Artificial Sequence
  primer
agagggatcctgtaattgttgaagttgctgcct

SEQ ID NO: 40 - DNA, 33 bp, Artificial Sequence
  primer
tgttgcggccgcttatggttctaatggtggatc

SEQ ID NO: 41 - DNA, 31 bp, Artificial Sequence
  primer
gtgtggatccatgacatatccaagaagaaga

SEQ ID NO: 42 - DNA, 44 bp, Artificial Sequence
  primer
atcttcttcttggatatgtcatggcatcaggattatcaacatta

SEQ ID NO: 43 - DNA, 44 bp, Artificial Sequence
  primer
taatgttgataatcctgatgccatgacatatccaagaagaagat

SEQ ID NO: 44 - DNA, 31 bp, Artificial Sequence
  primer
atgagtggatccatgaaaattattaatattg

SEQ ID NO: 45 - DNA, 36 bp, Enterococcus faecalis
ctaagttattttattgaacatatatcgtactttatc